European Patent Application EP 4 703 371 A1, published March 4, 2026. Title: Diagnostic and Therapeutic Properties of Peptide Epitopes Derived from Bullous Pemphigoid Extracellular Matrix Adhesion Proteins. Applicant: SeraDiaLogistics. The sequence listing filed with the application follows.

SEQUENCE LISTING (17 sequences)

SEQ ID NO: 1 - protein, 25 aa, synthetic construct
  source 1..25: note = BP 180 aa 499-522
VDELERIRRSILPYGDSMDRIEKDR

SEQ ID NO: 2 - protein, 15 aa, synthetic construct
  source 1..15: note = BP 180 aa 1316-1331
GGAGSLGAGGAFGEA

SEQ ID NO: 3 - protein, 15 aa, synthetic construct
  source 1..15: note = BP 180 aa 1456-1471
GPAGPPGHPGPPGPR

SEQ ID NO: 4 - protein, 15 aa, synthetic construct
  source 1..15: note = BP 230 aa 2432-2447
EGLITLTELADSLLS

SEQ ID NO: 5 - protein, 15 aa, synthetic construct
  source 1..15: note = BP 230 aa 2567-2582
EFQYLTGGLIEPQVH

SEQ ID NO: 6 - protein, 15 aa, synthetic construct
  source 1..15: note = BP 230 aa 2389-2402
SSHMLTDTKTGLHFN

SEQ ID NO: 7 - protein, 15 aa, synthetic construct
  source 1..15: note = BP 180 aa 1212-1227
FIPGPPGPPGPPGPR

SEQ ID NO: 8 - protein, 15 aa, synthetic construct
  source 1..15: note = BP 230 aa 2413-2428
INEAIEQGTIDKALV

SEQ ID NO: 9 - protein, 16 aa, synthetic construct
  source 1..16: note = BP 180 aa 1326-1342
AFGEAAGDRGPYGTDI

SEQ ID NO: 10 - protein, 15 aa, synthetic construct
  source 1..15: note = BP 230 aa 2434-2449
LITLTELADSLLSRL

SEQ ID NO: 11 - protein, 72 aa, synthetic construct
  source 1..72: note = BP 180 aa 491-562
EVRKLKARVDEVRKLKARVDPYGDSMDRIEKDRLQGMAPAAGADLDKIGLHSDSQEELWMFVRKKLMMEQEN

SEQ ID NO: 12 - protein, 307 aa, synthetic construct
  source 1..307: note = BP 180 aa 1191-1497
NVWSSISVEDLSSYLHTAGLSFIPGPPGPPGPPGPRGPPGVSGALATYAAENSDSFRSELISYLTSPDVRSFIVGPPGPPGPQGPPGDSRLLSTDASHSRGSSSSSHSSSVRRGSSYSSSMSTGGGGAGSLGAGGAFGEAAGDRGPYGTDIGPGGGYGAAAEGGMYAGNGGLLGADFAGDLDYNELAVRVSESMQRQGLLQGMAYTVQGPPGQPGPQGPPGISKVFSAYSNVTADLMDFFQTYGAIQGPPGQKGEMGTPGPKGDRGPAGPPGHPGPPGPRGHKGEKGDKGDQVYAGRRRRRSIAVKP

SEQ ID NO: 13 - protein, 331 aa, synthetic construct
  source 1..331: note = BP 230 aa 2329-2649
FLFPFGERNISNLNVKKTHRISVVDTKTGSELTVYEAFQRNLIEKSIYLELSGQQYQWKEAMFFESYGHSSHMLTDTKTGLHFNINEAIEQGTIDKALVKKYQEGLITLTELADSLLSRLVPKKDLHSPVAGYWLTASGERISVLKASRRNLVDRITALRCLEAQVSTGGIIDPLTGKKYRVAEALHRGLVDEGFAQQLRQCELVITGIGHPITNKMMSVVEAVNANIINKEMGIRCLEFQYLTGGLIEPQVHSRLSIEEALQVGIIDVLIATKLKDQKSYVRNIICPQTKRKLTYKEALEKADFDFHTGLKLLEVSEPLMTGISSLYYSS

SEQ ID NO: 14 - protein, 18 aa, synthetic construct
  source 1..18: note = NC16A peptide
RIRRSILPYGDSMDRIEK

SEQ ID NO: 15 - protein, 7 aa, synthetic construct
  source 1..7: note = artificial linker peptide
GSGSGSG

SEQ ID NO: 16 - protein, 10 aa, synthetic construct
  source 1..10: note = HA derived peptide
YPYDVPDYAG

SEQ ID NO: 17 - protein, 14 aa, synthetic construct
  source 1..14: note = polio derived peptide
KEVPALTAVETGAT